European Patent Specification EP 3 556 203 B1, published October 18, 2023. Title: Novel Brassica plants resistant to disease. Applicant: SYNGENTA PARTICIPATIONS AG Linders, Rico Briggs, Bill Wijnker, Thaam van der Ploeg, Sjaak. The sequence listing filed with the application follows.

SEQUENCE LISTING (6 sequences)

SEQ ID NO: 1 - DNA, 37 bp, Artificial
  Forward primer
cacgacgttgtaaaacgacaagagaattgtgcgctgc

SEQ ID NO: 2 - DNA, 36 bp, Artificial
  Reverse primer
caggaaacagctatgaccaaaagctgccacgaacac

SEQ ID NO: 3 - DNA, 23 bp, Artificial
  Forward primer
caccatctaggctctccccgagc

SEQ ID NO: 4 - DNA, 29 bp, Artificial
  Reverse primer
ggagccaagaatacaaatattgtatgtac

SEQ ID NO: 5 - DNA, 21 bp, Artificial
  Resistant specific probe
tcatgtttcgtcctagtatac

SEQ ID NO: 6 - DNA, 20 bp, Artificial
  Susceptible specific probe
ctaatcatgtttcgttcttc